European Patent Specification EP 3 481 415 B1, published September 6, 2023. Title: FIBRINOGENE LIQUIDE STABLE. Applicant: LABORATOIRE FRANCAIS DU FRACTIONNEMENT ET DES BIOTECHNOLOGIES. The sequence listing filed with the application follows.

SEQUENCE LISTING (95 sequences)

SEQ ID NO: 1 - DNA, 76 bp, Artificial
  Aptamer
gggtcaatgccaggtctcggacctggaatccgccacccgcattagaaccagggttgacatcggctcgcaagcagtc

SEQ ID NO: 2 - DNA, 76 bp, Artificial
  Aptamer
gggtcaatgccaggtctcggacctggaatccgccacccgcactagaaccagggttgacatcggctcgcaagcagtc

SEQ ID NO: 3 - DNA, 75 bp, Artificial
  Aptamer
gggtcaatgccaggtctcggacctggaatccgccacccgcattagaaccagggttgacatcggctcgcagcagtc

SEQ ID NO: 4 - DNA, 74 bp, Artificial
  Aptamer
gggtcaatgccaggtctcggacctggaatccgccacccgcattagaaccagggttgacatcggctcgcgcagtc

SEQ ID NO: 5 - DNA, 75 bp, Artificial
  Aptamer
gggtcaatgccaggtctcggacctggaatccgccacccgcattagaaccagggttgacatcggctcgcaagcagc

SEQ ID NO: 6 - DNA, 76 bp, Artificial
  Aptamer
gggtcaatgccaggtctcggacctggaatccgccacccgcattagaaccagggttgacgtcggctcgcaagcagtc

SEQ ID NO: 7 - DNA, 76 bp, Artificial
  Aptamer
gggtcaatgccaggtctcagacctggaatccgccacccgcattagaaccagggttgacatcggctcgcaagcagtc

SEQ ID NO: 8 - DNA, 76 bp, Artificial
  Aptamer
gggtcaatgccaggtctcggacctggaatccgccacccgcattaaaaccagggttgacatcggctcgcaagcagtc

SEQ ID NO: 9 - DNA, 76 bp, Artificial
  Aptamer
gggtcaatgccaggtctcggacctggaatccgtcacccgcattagaaccagggttgacatcggctcgcaagcagtc

SEQ ID NO: 10 - DNA, 76 bp, Artificial
  Aptamer
gggtcaatgccaggtctcggacctggaatccgccacccgcattagaaccagggttgacatcggctcgcaagcggtc

SEQ ID NO: 11 - DNA, 76 bp, Artificial
  Aptamer
gggtcaatgccaggtctcggacccggaatccgccacccgcattagaaccagggttgacatcggctcgcaagcagtc

SEQ ID NO: 12 - DNA, 76 bp, Artificial
  Aptamer
gggtcaatgccaggtctcggacctggaatccgccacccgcattagaaccagggttgacatcgactcgcaagcagtc

SEQ ID NO: 13 - DNA, 75 bp, Artificial
  Aptamer
gggtcaatgccaggtctcggacctggaatccgccacccgcactagaaccagggttgacatcggctcgcaagcatc

SEQ ID NO: 14 - DNA, 75 bp, Artificial
  Aptamer
gggtcaatgccaggtctcggacctggaatccgccacccgcactagaaccagggttgacatcggctcgcaagcgtc

SEQ ID NO: 15 - DNA, 76 bp, Artificial
  Aptamer
gggtcaatgccaggtctcggacccggaatccgccacccgcactagaaccagggttgacatcggctcgcaagcagtc

SEQ ID NO: 16 - DNA, 76 bp, Artificial
  Aptamer
gggtcaatgccaggtctcggaccaggaatccgccacccgcactagaaccagggttgacatcggctcgcaagcagtc

SEQ ID NO: 17 - DNA, 75 bp, Artificial
  Aptamer
gggtcaatgccaggtctcggacctggaatccgccacccgcactagaaccagggttgacatcggctgcaagcagtc

SEQ ID NO: 18 - DNA, 76 bp, Artificial
  Aptamer
gggtcaatgccaggtctcggacctggaatccgccacccgcactagagccagggttgacatcggctcgcaagcagtc

SEQ ID NO: 19 - DNA, 76 bp, Artificial
  Aptamer
gggtcaatgccaggtctcggacctggaatccgccacccgcactagaaccagggttgacatcggctcacaagcagtc

SEQ ID NO: 20 - DNA, 75 bp, Artificial
  Aptamer
gggtcaatgccaggtctcggacctggaatccgccacccgcactagaaccagggttgacatcggctccaagcagtc

SEQ ID NO: 21 - DNA, 74 bp, Artificial
  Aptamer
gggtcaatgccaggtctcggacctggaatccgccacccgcactagaaccagggttgacatcggctcaagcagtc

SEQ ID NO: 22 - DNA, 76 bp, Artificial
  Aptamer
gggtcaatgccaggtctcggacctggaatccgccacccgcactagaaccagggttgacatcggctcggaagcagtc

SEQ ID NO: 23 - DNA, 75 bp, Artificial
  Aptamer
gggtcaatgccaggtctcggacctggaatccgccacccgcactagaaccagggttgacatcggctcgaagcagtc

SEQ ID NO: 24 - DNA, 75 bp, Artificial
  Aptamer
gggtcaatgccaggtctcggacctggaatccgccacccgcactagaaccagggttgacatcggctcgcagcagtc

SEQ ID NO: 25 - DNA, 74 bp, Artificial
  Aptamer
gggtcaatgccaggtctcggacctggaatccgccacccgcactagaaccagggttgacatcggctcgcgcagtc

SEQ ID NO: 26 - DNA, 76 bp, Artificial
  Aptamer
gggtcaatgccaggtctcggacctggaatccgccacccgcactagaaccagggttgacatgggctcgcaagcagtc

SEQ ID NO: 27 - DNA, 74 bp, Artificial
  Aptamer
gggtcaatgccaggtctcggacctggaatccgccacccgcactagaaccagggttgacatcggctcgcacagtc

SEQ ID NO: 28 - DNA, 75 bp, Artificial
  Aptamer
gggtcaatgccaggtctcggacctggaatccgccacccgcactagaaccagggttgacatcggctcgcaacagtc

SEQ ID NO: 29 - DNA, 76 bp, Artificial
  Aptamer
gggtcaatgccaggtctcggacctggaatccgccacccgcactagaaccagggttgacatcagctcgcaagcagtc

SEQ ID NO: 30 - DNA, 76 bp, Artificial
  Aptamer
gggtcaatgccaggtctcggacctggaatccgccacccgcactagaaccagggctgacatcggctcgcaagcagtc

SEQ ID NO: 31 - DNA, 76 bp, Artificial
  Aptamer
gggtcaatgccaggtctcggacctggaatccgccacccgcattagaaccagggctgacatcggctcgcaagcagtc

SEQ ID NO: 32 - DNA, 76 bp, Artificial
  Aptamer
gggtcaatgccaggtctcggacctggaatccgccacccgcactagaaccagggttggcatcggctcgcaagcagtc

SEQ ID NO: 33 - DNA, 76 bp, Artificial
  Aptamer
gggtcaatgccaggtctcggacctggaatccgccacccgcattagaaccagggttggcatcggctcgcaagcagtc

SEQ ID NO: 34 - DNA, 76 bp, Artificial
  Aptamer
gggtcaatgccaggtctcggacctgggatccgccacccgcactagaaccagggttgacatcggctcgcaagcagtc

SEQ ID NO: 35 - DNA, 76 bp, Artificial
  Aptamer
gggtcaatgccaggtctcggacctgggatccgccacccgcattagaaccagggttgacatcggctcgcaagcagtc

SEQ ID NO: 36 - DNA, 76 bp, Artificial
  Aptamer
gggtcaatgccaggtctcggacctggaatccgccacccgcactagaaccagggttgacatcgggtcgcaagcagtc

SEQ ID NO: 37 - DNA, 76 bp, Artificial
  Aptamer
gggtcaatgccaggtctcggacctggaatccgccacccgcattagaaccagggttgacatcgggtcgcaagcagtc

SEQ ID NO: 38 - DNA, 76 bp, Artificial
  Aptamer
gggtcaatgccaggtctcggacctggaatccgccacccgcattagaaccagggtcgacatcggctcgcaagcagtc

SEQ ID NO: 39 - DNA, 76 bp, Artificial
  Aptamer
gggtcaatgccaggtctcggacctggaatccgccacccgcactagaaccagggtcgacatcggctcgcaagcagtc

SEQ ID NO: 40 - DNA, 76 bp, Artificial
  Aptamer
gggtcaatgccaggtctcgggcctggaatccgccacccgcattagaaccagggttgacatcggctcgcaagcagtc

SEQ ID NO: 41 - DNA, 76 bp, Artificial
  Aptamer
gggtcaatgccaggtctcgggcctggaatccgccacccgcactagaaccagggttgacatcggctcgcaagcagtc

SEQ ID NO: 42 - DNA, 76 bp, Artificial
  Aptamer
gggtcaatgccaggtctcggacctggaatccgccgcccgcattagaaccagggttgacatcggctcgcaagcagtc

SEQ ID NO: 43 - DNA, 76 bp, Artificial
  Aptamer
gggtcaatgccaggtctcggacctggaatccgccgcccgcactagaaccagggttgacatcggctcgcaagcagtc

SEQ ID NO: 44 - DNA, 76 bp, Artificial
  Aptamer
gggtcaatgccaggtctcggacctggaatccgcctcccgcattagaaccagggttgacatcggctcgcaagcagtc

SEQ ID NO: 45 - DNA, 76 bp, Artificial
  Aptamer
gggtcaatgccaggtctcggacctggaatccgccacccgcattagaaccagggttgacatcggctggcaagcagtc

SEQ ID NO: 46 - DNA, 74 bp, Artificial
  Aptamer
gggtcaatgccaggtctcggacctggaatccgccacccgcattagaaccagggttgacatcggctcaagcagtc

SEQ ID NO: 47 - DNA, 76 bp, Artificial
  Aptamer
gggtcaatgccaggtctcggacctggaatccgccacccgcattagaaccagggttgacatcggctcacaagcagtc

SEQ ID NO: 48 - DNA, 75 bp, Artificial
  Aptamer
gggtcaatgccaggtctcggacctggaatccgccacccgcattagaaccagggttgacatcggctcgaagcagtc

SEQ ID NO: 49 - DNA, 76 bp, Artificial
  Aptamer
gggtcaatgccaggtctcggacctggaatccgccacccgcattagaaccagggttgacatcggctcggaagcagtc

SEQ ID NO: 50 - DNA, 76 bp, Artificial
  Aptamer
gggtcaatgccaggtctcggacctggaatccgccacccgcattagaaccagggttgacatcggctcgcaaggagtc

SEQ ID NO: 51 - DNA, 76 bp, Artificial
  Aptamer
gggtcaatgccaggtctcggacctggaatccaccacccgcattagaaccagggttgacatcggctcgcaagcagtc

SEQ ID NO: 52 - DNA, 76 bp, Artificial
  Aptamer
gggtcaatgccaggtctcggacctggaatccgccacccgcattagaaccggggttgacatcggctcgcaagcagtc

SEQ ID NO: 53 - DNA, 75 bp, Artificial
  Aptamer
gggtcaatgccaggtctcggacctggaatccgccacccgcattagaaccagggttgacatcggctcgcaacagtc

SEQ ID NO: 54 - DNA, 76 bp, Artificial
  Aptamer
gggtcaatgccaggtctcgaacctggaatccgccacccgcattagaaccagggttgacatcggctcgcaagcagtc

SEQ ID NO: 55 - DNA, 76 bp, Artificial
  Aptamer
gggtcaatgccaggtctcgtacctggaatccgccacccgcattagaaccagggttgacatcggctcgcaagcagtc

SEQ ID NO: 56 - DNA, 76 bp, Artificial
  Aptamer
gggtcaatgccaggtctcggacctggaatccgccacccgcattagatccagggttgacatcggctcgcaagcagtc

SEQ ID NO: 57 - DNA, 76 bp, Artificial
  Aptamer
gggtcaatgccaggtctcggacctggaatccgccacccgcattaggaccagggttgacatcggctcgcaagcagtc

SEQ ID NO: 58 - DNA, 76 bp, Artificial
  Aptamer
gggtcaatgccaggtctcaactttcgcgtgtggttggtagggctaggtgtatacgcatatcggctcgcaagcagtc

SEQ ID NO: 59 - DNA, 75 bp, Artificial
  Aptamer
gggtcaatgccaggtctcaggtgagtcttacggatgtggttggtagggctaggtgtatatcggctcgcaagcagt

SEQ ID NO: 60 - DNA, 76 bp, Artificial
  Aptamer
gggtcaatgccaggtctctgcgtacttatctcgatgtggttggtagggataggtgtatatcggctcgcaagcagtc

SEQ ID NO: 61 - DNA, 74 bp, Artificial
  Aptamer
gggtcaatgccaggtctcgatctctgtggttggtaggggagtgtgtatagtgtcgtatcggctcgcaagcagtc

SEQ ID NO: 62 - DNA, 75 bp, Artificial
  Aptamer
gggtcaatgccaggtctcgctgtggttggtagggataggtgtatggcagctggataggatcggctcgcaagcagt

SEQ ID NO: 63 - DNA, 75 bp, Artificial
  Aptamer
gggtcaatgccaggtctcaataaaagtagctgatgtgcgttggtagggaacggtgtatatcggctcgcaagcagt

SEQ ID NO: 64 - DNA, 75 bp, Artificial
  Aptamer
gggtcaatgccaggtctcggcgtagaagccggaatgtggttggtagggttaggtgtatatcggctcgcaagcagt

SEQ ID NO: 65 - DNA, 76 bp, Artificial
  Aptamer
gggtcaatgccaggtctcgagccggtgttgtgttatgttggtagggaaggtgtataatatcggctcgcaagcagtc

SEQ ID NO: 66 - DNA, 58 bp, Artificial
  Core sequence A.5-1.9
gggtcaatgccaggtctcggacctggaatccgccacccgcattagaaccagggttgac

SEQ ID NO: 67 - DNA, 34 bp, Artificial
  Core sequence A5-2.9
cgcgtgtggttggtagggctaggtgtatacgcat

SEQ ID NO: 68 - DNA, 40 bp, Artificial
  Central region
aggtgagtcttacggatgtggttggtagggctaggtgtat

SEQ ID NO: 69 - DNA, 40 bp, Artificial
  Central region
tgcgtacttatctcgatgtggttggtagggataggtgtat

SEQ ID NO: 70 - DNA, 38 bp, Artificial
  Central region
gatctctgtggttggtaggggagtgtgtatagtgtcgt

SEQ ID NO: 71 - DNA, 40 bp, Artificial
  Central region
gctgtggttggtagggataggtgtatggcagctggatagg

SEQ ID NO: 72 - DNA, 40 bp, Artificial
  Central region
aataaaagtagctgatgtgcgttggtagggaacggtgtat

SEQ ID NO: 73 - DNA, 40 bp, Artificial
  Central region
ggcgtagaagccggaatgtggttggtagggttaggtgtat

SEQ ID NO: 74 - DNA, 40 bp, Artificial
  Central region
gagccggtgttgtgttatgttggtagggaaggtgtataat

SEQ ID NO: 75 - DNA, 18 bp, Artificial
  Primer
gggtcaatgccaggtctc

SEQ ID NO: 76 - DNA, 18 bp, Artificial
  Primer
atcggctcgcaagcagtc

SEQ ID NO: 77 - DNA, 10 bp, Artificial
  consensus moiety
gttggtaggg

SEQ ID NO: 78 - DNA, 7 bp, Artificial
  Consensus moiety
ggtgtat

SEQ ID NO: 79 - DNA, 3 bp, Artificial
  consensus moiety
tgt

SEQ ID NO: 80 - DNA, 56 bp, Artificial
  Aptamer
gtcaatgccaggtctcggacctggaatccgccacccgcattagaaccagggttgac

SEQ ID NO: 81 - DNA, 53 bp, Artificial
  Aptamer
gtcaatgccaggtctccctggaatccgccacccgcattagaaccagggttgac

SEQ ID NO: 82 - DNA, 50 bp, Artificial
  Aptamer
gtcaatgccagtcgctggaatccgccacccgcattagaaccagggttgac

SEQ ID NO: 83 - DNA, 52 bp, Artificial
  Aptamer
gtcaatgccaggtctcctggaatccgccacccgcattagaaccagggttgac

SEQ ID NO: 84 - DNA, 52 bp, Artificial
  Aptamer
gtcaatgccaggtcacctggaatccgccacccgcattagaaccagggttgac

SEQ ID NO: 85 - DNA, 53 bp, Artificial
  Aptamer
gtcaatgccaggtcgacctggaatccgccacccgcattagaaccagggttgac

SEQ ID NO: 86 - DNA, 52 bp, Artificial
  Aptamer
gtcaatgccaggtcgcctggaatccgccacccgcattagaaccagggttgac

SEQ ID NO: 87 - DNA, 54 bp, Artificial
  Aptamer
gtcaatgccaggtctcacctggaatccgccacccgcattagaaccagggttgac

SEQ ID NO: 88 - DNA, 54 bp, Artificial
  Aptamer
gtcaatgccaggtcggacctggaatccgccacccgcattagaaccagggttgac

SEQ ID NO: 89 - DNA, 55 bp, Artificial
  Aptamer
gtcaatgccaggtctcggacctggaatccgccacccgcattagaaccagggttga

SEQ ID NO: 90 - DNA, 55 bp, Artificial
  Aptamer
gtcaatgccaggtctcggacctggaatccgccacccgcatagaaccagggttgac

SEQ ID NO: 91 - DNA, 53 bp, Artificial
  Aptamer
gtcaatgccagtcggacctggaatccgccacccgcattagaaccagggttgac

SEQ ID NO: 92 - DNA, 55 bp, Artificial
  Aptamer
gtcaatgccaggtctcggacctggaatccgccacccgcttagaaccagggttgac

SEQ ID NO: 93 - DNA, 52 bp, Artificial
  Aptamer
gtcaatgccagcggacctggaatccgccacccgcattagaaccagggttgac

SEQ ID NO: 94 - DNA, 40 bp, Artificial
  central region
ggacctggaatccgccacccgcattagaaccagggttgac

SEQ ID NO: 95 - DNA, 40 bp, Artificial
  central region
aactttcgcgtgtggttggtagggctaggtgtatacgcat